European Patent Application EP 4 219 537 A1, published August 2, 2023. Title: GLYCOSYLATION-MODIFIED ERYTHOPOIETIN AND USE THEREOF. Applicant: JECHO BIOPHARMACEUTICALS CO., LTD.; JECHO LABORATORIES, INC.; JECHO INSTITUTE, CO., LTD. The sequence listing filed with the application follows.

SEQUENCE LISTING (4 sequences)

SEQ ID NO: 1 - protein, 165 aa, Artificial Sequence
  EPO
APPRLICDSRVLERYLLEAKEAENITTGCNETCSLNENITVPDTKVNFYAWKRMEVGQQAVEVWQGLALLSEAVLRGQALLVNSSQVNETLQLHVDKAVSGLRSLTTLLRALGAQKEAISPPDAASAAPLRTITADTFRKLFRVYSNFLRGKLKLYTGEACRTGD

SEQ ID NO: 2 - DNA, 60 bp, Homo sapiens
atgtacaggatgcaactcctgtcttgcattgcactaagtcttgcacttgtcacaaacagt

SEQ ID NO: 3 - DNA, 7791 bp, Artificial Sequence
  JL14001
tcaatattggccattagccatattattcattggttatatagcataaatcaatattggctattggccattgcatacgttgtatctatatcataatatgtacatttatattggctcatgtccaatatgaccgccatgttggcattgattattgactagttattaatagtaatcaattacggggtcattagttcatagcccatatatggagttccgcgttacataacttacggtaaatggcccgcctggctgaccgcccaacgacccccgcccattgacgtcaataatgacgtatgttcccatagtaacgccaatagggactttccattgacgtcaatgggtggagtatttacggtaaactgcccacttggcagtacatcaagtgtatcatatgccaagtccgccccctattgacgtcaatgacggtaaatggcccgcctggcattatgcccagtacatgaccttacgggactttcctacttggcagtacatctacgtattagtcatcgctattaccatggtgatgcggttttggcagtacaccaatgggcgtggatagcggtttgactcacggggatttccaagtctccaccccattgacgtcaatgggagtttgttttggcaccaaaatcaacgggactttccaaaatgtcgtaacaactgcgatcgcccgccccgttgacgcaaatgggcggtaggcgtgtacggtgggaggtctatataagcagagctcgtttagtgaaccgtcagatcactagaagctttattgcggtagtttatcacagttaaattgctaacgcagtcagtgcttctgacacaacagtctcgaacttaagctgcagtgactctcttaaggtagccttgcagaagttggtcgtgaggcactgggcaggtaagtatcaaggttacaagacaggtttaaggagaccaatagaaactgggcttgtcgagacagagaagactcttgcgtttctgataggcacctattggtcttactgacatccactttgcctttctctccacaggtgtccactcccagttcaattacagctcttaaggctagagtacttaatacgactcactataggctagccgccaccatgtacaggatgcaactcctgtcttgcattgcactaagtcttgcacttgtcacaaacagtgccccaccacgcctcatctgtgacagccgagtcctggagaggtacctcttggaggccaaggaggccgagaatatcacgacgggctgtaatgaaacctgcagcttgaatgagaatatcactgtcccagacaccaaagttaatttctatgcctggaagaggatggaggtcgggcagcaggccgtagaagtctggcagggcctggccctgctgtcggaagctgtcctgcggggccaggccctgttggtcaactcttcccaggtgaatgagaccctgcagctgcatgtggataaagccgtcagtggccttcgcagcctcaccactctgcttcgggctctgggagcccagaaggaagccatctcccctccagatgcggcctcagctgctccactccgaacaatcactgctgacactttccgcaaactcttccgagtctactccaatttcctccggggaaagctgaagctgtacacaggggaggcctgcaggacaggggactaactcgagaattcacgcgtcgagcatgcatctagggcggccaattccgcccctctcccccccccccctctccctcccccccccctaacgttactggccgaagccgcttggaataaggccggtgtgcgtttgtctatatgttattttccaccatattgccgtcttttggcaatgtgagggcccggaaacctggccctgtcttcttgacgagcattcctaggggtctttcccctctcgccaaaggaatgcaaggtctgttgaatgtcgtgaaggaagcagttcctctggaagcttcttgaagacaaacaacgtctgtagcgaccctttgcaggcagcggaaccccccacctggcgacaggtgcctctgcggccaaaagccacgtgtataagatacacctgcaaaggcggcacaaccccagtgccacgttgtgagttggatagttgtggaaagagtcaaatggctctcctcaagcgtattcaacaaggggctgaaggatgcccagaaggtaccccattgtatgggatctgatctggggcctcggtgcacatgctttacatgtgtttagtcgaggttaaaaaaacgtctaggccccccgaaccacggggacgtggttttcctttgaaaaacacgatgataagcttgccacaacccgggatcctctagagccgccaccatggccacctcagcaagttcccacttgaacaaaggcatcaagcagatgtacatgaacctgccccagggcgagaagatccaactcatgtatatctgggttgatggtaccggggaagggctacgctgcaagacccgtactctggactgtgaccccaagtgtgtagaagagttacccgagtggaactttgatggttctagtacgtttcagtctgaaggctccaacagcggcatgtacctccatcctgtggccatgtttcgagaccccttccgcagagaccccaacaagctggtgttctgcgaagtattcaagtataaccggaagcccgcagagaccaacctgaggcacagctgtaagcgtataatggacatggtgagcagccagcacccctggtttggaatggaacaggagtatactctcatgggaacagacggccaccctttcggctggccttctaatggcttccctggaccccaaggaccctattactgcggtgtgggagctgacaaggcttatggccgagatatcgtggaggctcactaccgggcctgcttgtatgctggaatcaagatcacagggacaaatgccgaggttatgcctgcccagtgggaattccagataggaccctgcgaagggatccgcatgggagatcatctctgggtagcccgttttatcttgcatcgggtatgcgaagactttggggtgatagcaacctttgaccccaagcccattccagggaactggaatggggcaggctgccacaccaactttagcaccaaggccatgcgggaggagaatggtctgaggtgcattgaggaggccattgataaactgagcaagaggcaccagtaccacatccgtgcctacgaccccaaggggggcctggacaacgcccgccgtctgactggattccacgaaacctccaacatcaacgacttttccgctggcgttgccaaccgcagcgccagtatccgcattccccggattgtcggccaggagaagaagggttactttgaagaccgtcggccttctgccaattgcgacccctatgcggtgacggaagccatcgtccgcacgtgtctcctcaacgaaactggcgacgagcccttccaatacaagaactaagcggccgcttccctttagtgagggttaatgcttcgagcagacatgataagatacattgatgagtttggacaaaccacaactagaatgcagtgaaaaaaatgctttatttgtgaaatttgtgatgctattgctttatttgtaaccattataagctgcaataaacaagttaacaacaacaattgcattcattttatgtttcaggttcagggggagatgtgggaggttttttaaagcaagtaaaacctctacaaatgtggtaaaatccgataaggatcgatccgggctggcgtaatagcgaagaggcccgcaccgatcgcccttcccaacagttgcgcagcctgaatggcgaatggacgcgccctgtagcggcgcattaagcgcggcgggtgtggtggttacgcgcagcgtgaccgctacacttgccagcgccctagcgcccgctcctttcgctttcttcccttcctttctcgccacgttcgccggctttccccgtcaagctctaaatcgggggctccctttagggttccgatttagtgctttacggcacctcgaccccaaaaaacttgattagggtgatggttcacgtagtgggccatcgccctgatagacggtttttcgccctttgacgttggagtccacgttctttaatagtggactcttgttccaaactggaacaacactcaaccctatctcggtctattcttttgatttataagggattttgccgatttcggcctattggttaaaaaatgagctgatttaacaaaaatttaacgcgaattttaacaaaatattaacgcttacaatttcctgatgcggtattttctccttacgcatctgtgcggtatttcacaccgcatacgcggatctgcgcagcaccatggcctgaaataacctctgaaagaggaacttggttaggtaccttctgaggcggaaagaaccagctgtggaatgtgtgtcagttagggtgtggaaagtccccaggctccccagcaggcagaagtatgcaaagcatgcatctcaattagtcagcaaccaggtgtggaaagtccccaggctccccagcaggcagaagtatgcaaagcatgcatctcaattagtcagcaaccatagtcccgcccctaactccgcccatcccgcccctaactccgcccagttccgcccattctccgccccatggctgactaattttttttatttatgcagaggccgaggccgcctcggcctctgagctattccagaagtagtgaggaggcttttttggaggcctaggcttttgcaaaaagcttgattcttctgacacaacagtctcgaacttaaggctagagccaccatgattgaacaagatggattgcacgcaggttctccggccgcttgggtggagaggctattcggctatgactgggcacaacagacaatcggctgctctgatgccgccgtgttccggctgtcagcgcaggggcgcccggttctttttgtcaagaccgacctgtccggtgccctgaatgaactgcaggacgaggcagcgcggctatcgtggctggccacgacgggcgttccttgcgcagctgtgctcgacgttgtcactgaagcgggaagggactggctgctattgggcgaagtgccggggcaggatctcctgtcatctcaccttgctcctgccgagaaagtatccatcatggctgatgcaatgcggcggctgcatacgcttgatccggctacctgcccattcgaccaccaagcgaaacatcgcatcgagcgagcacgtactcggatggaagccggtcttgtcgatcaggatgatctggacgaagagcatcaggggctcgcgccagccgaactgttcgccaggctcaaggcgcgcatgcccgacggcgaggatctcgtcgtgacccatggcgatgcctgcttgccgaatatcatggtggaaaatggccgcttttctggattcatcgactgtggccggctgggtgtggcggaccgctatcaggacatagcgttggctacccgtgatattgctgaagagcttggcggcgaatgggctgaccgcttcctcgtgctttacggtatcgccgctcccgattcgcagcgcatcgccttctatcgccttcttgacgagttcttctgagcgggactctggggttcgaaatgaccgaccaagcgacgcccaacctgccatcacgatggccgcaataaaatatctttattttcattacatctgtgtgttggttttttgtgtgaatcgatagcgataaggatccgcgtatggtgcactctcagtacaatctgctctgatgccgcatagttaagccagccccgacacccgccaacacccgctgacgcgccctgacgggcttgtctgctcccggcatccgcttacagacaagctgtgaccgtctccgggagctgcatgtgtcagaggttttcaccgtcatcaccgaaacgcgcgagacgaaagggcctcgtgatacgcctatttttataggttaatgtcatgataataatggtttcttagacgtcaggtggcacttttcggggaaatgtgcgcggaacccctatttgtttatttttctaaatacattcaaatatgtatccgctcatgagacaataaccctgataaatgcttcaataatattgaaaaaggaagagtatgagtattcaacatttccgtgtcgcccttattcccttttttgcggcattttgccttcctgtttttgctcacccagaaacgctggtgaaagtaaaagatgctgaagatcagttgggtgcacgagtgggttacatcgaactggatctcaacagcggtaagatccttgagagttttcgccccgaagaacgttttccaatgatgagcacttttaaagttctgctatgtggcgcggtattatcccgtattgacgccgggcaagagcaactcggtcgccgcatacactattctcagaatgacttggttgagtactcaccagtcacagaaaagcatcttacggatggcatgacagtaagagaattatgcagtgctgccataaccatgagtgataacactgcggccaacttacttctgacaacgatcggaggaccgaaggagctaaccgcttttttgcacaacatgggggatcatgtaactcgccttgatcgttgggaaccggagctgaatgaagccataccaaacgacgagcgtgacaccacgatgcctgtagcaatggcaacaacgttgcgcaaactattaactggcgaactacttactctagcttcccggcaacaattaatagactggatggaggcggataaagttgcaggaccacttctgcgctcggcccttccggctggctggtttattgctgataaatctggagccggtgagcgtgggtctcgcggtatcattgcagcactggggccagatggtaagccctcccgtatcgtagttatctacacgacggggagtcaggcaactatggatgaacgaaatagacagatcgctgagataggtgcctcactgattaagcattggtaactgtcagaccaagtttactcatatatactttagattgatttaaaacttcatttttaatttaaaaggatctaggtgaagatcctttttgataatctcatgaccaaaatcccttaacgtgagttttcgttccactgagcgtcagaccccgtagaaaagatcaaaggatcttcttgagatcctttttttctgcgcgtaatctgctgcttgcaaacaaaaaaaccaccgctaccagcggtggtttgtttgccggatcaagagctaccaactctttttccgaaggtaactggcttcagcagagcgcagataccaaatactgttcttctagtgtagccgtagttaggccaccacttcaagaactctgtagcaccgcctacatacctcgctctgctaatcctgttaccagtggctgctgccagtggcgataagtcgtgtcttaccgggttggactcaagacgatagttaccggataaggcgcagcggtcgggctgaacggggggttcgtgcacacagcccagcttggagcgaacgacctacaccgaactgagatacctacagcgtgagctatgagaaagcgccacgcttcccgaagggagaaaggcggacaggtatccggtaagcggcagggtcggaacaggagagcgcacgagggagcttccagggggaaacgcctggtatctttatagtcctgtcgggtttcgccacctctgacttgagcgtcgatttttgtgatgctcgtcaggggggcggagcctatggaaaaacgccagcaacgcggcctttttacggttcctggccttttgctggccttttgctcacatggctcgacagatct

SEQ ID NO: 4 - DNA, 1122 bp, Rattus norvegicus
atggccacctcagcaagttcccacttgaacaaaggcatcaagcagatgtacatgaacctgccccagggcgagaagatccaactcatgtatatctgggttgatggtaccggggaagggctacgctgcaagacccgtactctggactgtgaccccaagtgtgtagaagagttacccgagtggaactttgatggttctagtacgtttcagtctgaaggctccaacagcggcatgtacctccatcctgtggccatgtttcgagaccccttccgcagagaccccaacaagctggtgttctgcgaagtattcaagtataaccggaagcccgcagagaccaacctgaggcacagctgtaagcgtataatggacatggtgagcagccagcacccctggtttggaatggaacaggagtatactctcatgggaacagacggccaccctttcggctggccttctaatggcttccctggaccccaaggaccctattactgcggtgtgggagctgacaaggcttatggccgagatatcgtggaggctcactaccgggcctgcttgtatgctggaatcaagatcacagggacaaatgccgaggttatgcctgcccagtgggaattccagataggaccctgcgaagggatccgcatgggagatcatctctgggtagcccgttttatcttgcatcgggtatgcgaagactttggggtgatagcaacctttgaccccaagcccattccagggaactggaatggggcaggctgccacaccaactttagcaccaaggccatgcgggaggagaatggtctgaggtgcattgaggaggccattgataaactgagcaagaggcaccagtaccacatccgtgcctacgaccccaaggggggcctggacaacgcccgccgtctgactggattccacgaaacctccaacatcaacgacttttccgctggcgttgccaaccgcagcgccagtatccgcattccccggattgtcggccaggagaagaagggttactttgaagaccgtcggccttctgccaattgcgacccctatgcggtgacggaagccatcgtccgcacgtgtctcctcaacgaaactggcgacgagcccttccaatacaagaactaa